European Patent Application EP 4 170 033 A1, published April 26, 2023. Title: A transformant of hydrogenophilus genus for producing aspartate and methionine. Applicant: SUMITOMO CHEMICAL COMPANY, LIMITED Utilization of Carbon Dioxide Institute Co., Ltd. The sequence listing filed with the application follows.

SEQUENCE LISTING (44 sequences)

SEQ ID NO: 1 - DNA, 783 bp, Candidatus Hydrothermae bacterium
atgagagcagggattattggatgtggagccatcggatcattccttgccagagaaatcgacagaggcaatgtggctcacatgaaacttgttgcactgtttgatatagatttaaataaggtatataaacttgtggagtctttagaacataagcctcaaatagctgatagttttgagaaatttttaaaattacccgtggattttgtaatagaggcagcctcccagcaggcagtttttcagtatgcagaaaaaatcttaaagcaaaaaaaaccgcttcttcttatgagtgcaggtgctcttgcagatgatagattaagagaaaaattatttcgggtggctcgggaaaataataccaaaatttatattccctctggtgccattgcggggcttgacggcctcaaggcaatgagcaatgtgagacttcaccgtgcaagactcactacacgaaaatccccctctgcattgggggttaaaacggagaagcctgttgtggttttctcagggaatgcccatgaagcagccaaaagatatccccaaaatattaatgttgcgattgcatttggtctggctgctcatgccatagatatcctccaggtagagattgtagctgacccaggagtttcaaggaatatacacacaatagaagtagagggggaggctggaaaactggaaattacactggaaaattttcccttcccggacaatccaaaaacaagttttctcgcagcactttctgctcttcaggtgttaaaaaatatagcatccaatgtagtaattggaggttaa

SEQ ID NO: 2 - DNA, 792 bp, Glaciecola sp. 33A
atgattaaaattggcctaataggctttggtgcaatcggtcggtgtgtgatcgaaacactccccaaagcgttaactgaagaatatgaagttatcggtatcctaactagaaaagctgctgacaattgggtgaataatattccctcttatagcgatatagaccagttacttgcaaaacaacccgacattattgtcgaatgtgcgggtcatcatgcggttaaagaatatggttgtaaaatattagaagccaatatatcactcgttatatcatccattggtgccttagctgatagtgttttatatcaacaacttaaagattcatctacggctagtaaggcaaaaatatatctgccggctggcgccattggtggtattgatgcccttgttgccgcaaaacttggcgggattcacgatgtcacttataccatgcgaaagcctcccaaggcttggcaaggttcggttgctgagacggtggttgacttgaatagtcttaagcaggcaaccgttattttttctggctctgccggtgaagcagcaacactttaccctaaaaacaccaatgtaactgcaaccattgcgttagcgggattaggttttgatgagacaaaagtagaattaattgcagatcccaacattattgacaatatacacgaaatatcggtatccggtgaaacagggtattttaccattgtattaaaaggaaaaccctctgtgtataacccaaaaacttcagcattaacggcttttagtgtcactaagtgcgttgctgattttggctcatcgatcattatttaa

SEQ ID NO: 3 - DNA, 777 bp, Mesorhizobium sp. M7D.F.Ca.US.005.01.1.1
atggtcacgctcggcctcatcgggttcggcacgatctcgcgcgcgatcgtctccgctttcccaccggactcgtgtcgctgggtggcgctgatgcgcgaaggcgcccgccccgcactgccggcgaacgtcagcactgtcacgcagcttgacgcgctgatcagtgcgcgtccaagcacggtggtcgaggcggcaagtcaggaagcagtggccgcctacgtgcccgcgcttctcgacgccggcatcccgaccatcatcgcttcgatcggtgcgttctccgatccgatacttgccgcccggttaaccgatgcttcgcgcaacagcggcgcgcgcttggtcctgccgtcaggcgcgttgggcggcctcgactatctcagggcgatagcggcacttcccgatgcacgggtgcgctatacctcgcgcaagccgccggcagcctggaaagccgagcttgccactcttggcctatccgccgagcacgatgcggtatcgctcttcgagggcacgcccgcgcaagcggcaaaactctatccgaaaaacctcaacgccgccttcgccgtggcgctcgcggcaggcatcgacaaagtcaccgtgagcgtggttgccgatccgaaaactaccggcaacacgcacgagatcgaggtcgagagcaccgccggcaccgcctccttccgcctcgtcaacgcgccctcgcccagcaatccgaagacctcgatgctcacggcgctcagcctcgtcgcggcgcttagcgagttgctcgacagggagggctgtcactga

SEQ ID NO: 4 - DNA, 801 bp, Rhodospirillaceae bacterium
atgttgaatataggattattaggattaggagcaattggttcagatgttttaaatatggtgcgagaagaattttccaaccaaatccagataccagccgttttagtcaaacgcccccgcaaagaaaaacttatgggccattcattaatcaccaatgattttgaggagttttttagtaaagaacaagacattgttctagaagtagctggccactcgactgtgcggcattatggagaacgcatattgaaatctggagttgaccttatggtaacgtccgttggagctttcactgatgatactctatataaaagatgcatcaaagcagccacaacatctggttcacgtctaattatcccatctgcaggaatcggctctctggatactttgtcagccgccgcagtaggcggtttagattccgtgcacatgatagtcagaaaagatccaacagcttggtacggaacacatgctgaaaatttatttgatcttgctgcactaaaaaaacccaccataatttttgagggtagcccgagggaaggagccgctctgtatccacaaaacgttaatatttcagccgctgtatctctagcaggtatgggcctcgataaaacaagattaacgattatcgctgatacagaaattgacactcacgtctgtgagattcacgccaatggcgccttcggaagttatacctttagagaagatttaacagtcgccgaaactaaccgaaaaactggtaaaatcgttgccatggctgttatgaaaacaatacgccaaatggttagcccagtgttaataggcgtttga

SEQ ID NO: 5 - DNA, 783 bp, Bacillus kochii
atgaagctgggattaataggtggaggaaatatcggaaaatttttgctacaatctatcaatagcgataaattggtagatggcgcacaattcgttggattgtatacaagaaatcaagagaaagcaaatgagctggctgaagagtatgatttgcgaagctaccaatcaatcgatgaactgattgcttcagatatagatgtgatagttgaagcagctactgtagacgttgttcgagcccatgccacatcggttctcacacatggtaaagatcttgttgtgagcagtgttggcgcattttctgataacgactattttctccaattagaaacgatttgtaaagaacaagggacaacgattcatttaccttcaggtgcagtaggaggcttggatatattaaaagctgctaaggctattggtgctttacaagaagtatcgttaacaacaacgaagccaccgcatgccttaaacggtgttactctcgagaataaaacagtcttatttgaaggtaatgcctatgaagcgattaaacagtttcctaagaatattaacgtatcaattattctatcattagctggacttggttcaaaagagacaaaagtgaagattattgctgatccaaaagcaacgaaaaatagtcatgagattacagctaaaggggcgtttggaaaagtgaaactagtggttgaaaatgatccgatgccaaacaacccaaagacaagttacttagcagctttaagtgttctctcaacattgaaacataaggatcaatctatcaaagtggggtaa

SEQ ID NO: 6 - DNA, 774 bp, Novosphingobium rosa
atgctgcgcatcggatttatcggcaatggttccatcgcccgcgcggcctgcgcagcgctgggcccggatgtgacgctctgcggccatctggcccgtccggggcgtagcgatggcgatctggcggtcgagcggctggccgatctgctggaccgtcagcccgatgtggtggtggaatgcgccggccatgaggccgtgcgcgagcatggcgcggcggtgctggaggcgggcgtggcactgatggtggtgtccatcggcgcgctggccgatccggcattggaaagcgccttgaacgatgccgcgacccgcagcggcgcgcgcctgatccttcccgcaggcgcggtgggcggcatcgatgctctgacggcggccaagctgggcggcctgtccagcgtgacctatcgcgcgcgcaaaccggccatggcctgggcgggcagcccggccgagaaggtcgtggatctcgcttcccttggcgaggccacgaccttctttcgcggcaccgcgcgcgaggccgccatcgcttttcccaagaactccaatgtcgcggccacggtagcgctggctggcgtcggtttcgatgccacgcaggtcgagctggtcgccgatccacattcctcgcgcaacctgcacgagatctgcttcgagggggccgatggcgccttccgcttcgagatcgagggccgtccctcgcccgacaatcccaagacctcgctgctgaccgcgcatagcgtggcgcgcgaattgctcaccttcgccgcccagagaaaggcccgctga

SEQ ID NO: 7 - DNA, 711 bp, Archaeoglobus fulgidus
atgttagtcggcttaattggatacggggcaattggaaaatttctggctgagtggcttgaaaggaacggatttgagattgctgccattctggatgtaaggggagagcacgagaagatggttagaggcattgacgagttcctccagagggagatggatgtggccgttgaggctgcatcgcagcaagctgttaaggactatgcggagaaaattcttaaggctggcatagacctaattgttctgagcaccggggccttcgctgacagggattttctcagcagagtcagggaagtctgcaggaaaacgggcaggagagtttacatagcatctggggcaatcggtggattggatgccattttttcagcatcagagttgatagaggaaatcgttctgacaacaaggaagaattggaggcagtttggcagaaaaggtgtaatattcgaaggctctgcatctgaggcagctcagaaattcccgaaaaacttgaacgttgcagcgacgctcagcattgcctcaggaaaagacgtgaaggtcaggcttgtagctgacgaggttgaggagaacatccacgaaattctggtgaggggagagtttggggagatggaaatcagagttaggaacaggccaatgagggaaaatccgaagacgagctatcttgctgccctttctgtaacgagaattttgagaaatcttaaggagggattggtggtttga

SEQ ID NO: 8 - DNA, 810 bp, Arthrobacter sp. 161MFSha2.1
atgacgtcccaccgcataggaatcattggctacggagccatcggcgcgcgcgtcgccgaggacatctccctgggcaaggtggtgggcgcagaactggccggcatcatcagccgcaccgacaacggaaccgggcgtcccgccgtcgaacgccccttcccttcgctgaccttggaagcggccctggagtgctgcgagctgatcgtggagtgcgcggggcagtccgccgtgactgaatacgctgaaaagatcctgggcgcgggcgtagatttcctgatcacctccatcggcgcccttgccgaccaggacctggcagcacgcttgaacgcgtgcggtccagggagattgttcatgacgtcgggcgcagtgggcgggctcgacctccttgaagccggcgcaagggaagccgcctacgattccgtggtggtttccaccaccaaacttcctgaaacgctggtccaaccttggatggaacaggagcaagccgatgggatccgagcgaccacagaaccgctggaggtcttcctcggctcagcccaggaagcggcacggctgtttccgcgctcactcaacgtcgcagcggccgtggctgaggccgtcggggattgggacggcgtgcaggtgcggctgacggccgacccgaaggcctcactgaccagccacgtcattgaagcctcgggcccctccggcgaataccgcttcgagatccgcaacaaccccagtccgcagaacccgaggaccagcgggatagtcccctttgccgtcctccggtccttggaagcggcgatcggcgaacgcggagggctggtctag

SEQ ID NO: 9 - DNA, 762 bp, Oceanotoga teriensis
atgtttttattgaatattttttttattggggcaggaaattgtactgaaataattcttgaaaaaatgcagaattgtataaaaaaagcttatttattagattatgatgttgaaaaaattaattttttaaaagaaaaatttcatttttgtattgaatccgatttttttatttctgatgatattgatttttatgtggaatgtgcgagtgttgaagctgtgaaaaaatatactgaaaacataattaggaataataagaatattattattttatcaagtggcgctttttcagattttgattttcgaaacaatgttgaaaatattttaaaaaattcaaggtctcaaatatttattccatctggagctattggtggaattgatattattaattctttgaaagatgaaattaattctattactatagaaactcgtaaacccccattaagttttaatatgataaatacaaaagaagaacttattttttatggaactgccgaagaagctattaaaaattatcctaaaaatattaatgttgctatcactctttcaatggccgttgaaagttttgataaagttaaagtaaaaattatttctgatccaaaaataattaaaaatattcataaaatatttatagattcaaaagcaggtaaatatgaaataaaaattgaaaataatccttctaataatccaaaaacaagtttaatggcaccattatctgtagttggatttctaaaaaaatttaataatagtattaaggttggtgtttaa

SEQ ID NO: 10 - DNA, 756 bp, Marinitoga sp. 1155
atgttgaaagtatttcttttaggagcgggaaattctgcaaaaattattctggatgaattgaatttcgaaaaggtttatgtatatgataaaaatttcaagcaatttgaaaaactaaaagaaatacataatgaaatcgaatatttagatattaaaaacttagaaactactgatgttgattatattatagaagtagcatctgttgaagcattaaagaattatggactaaaactccttgatatgaataaaaatttaattgtcttaagtacaggcgcttttgcagataaaatttttagatataattttgtgaaaaaattaaataacaaaaatattaatgtttatgttgtatctggagcaatcggtggaattgatctaataagaaccataagcgataaaataaatacaatcacattaataacacgaaaaacaccaaaaagtcttgggattgatattaaaaaagaaaaaataatttttgaaggtaattcaatagaagctattgaaagattccctaaaaatataaatgttgctgttacgctggcattggcaataaaaaattttgaaaaggtaaaagttaaaattatagcagatccttttattgaaagaaatgtacattcaatagaaataaaatcaaaggttggaaattatacatttaaatttgaaaattatccatcaaaaaatccaaaaaccagttatctggcaccattatctatagttggattattgaaaaacattcactcaaaattcaaaataggaggataa

SEQ ID NO: 11 - DNA, 747 bp, Thermotogales bacterium 46_20
atggacaaaataagcgtactgctgatcggtggaggcaacatcgctcatatcctgctcaatgaacttggacacagaatcagaaaatcctactaccatgatctcagaaagacagatctggaggccacctttctggaatcctttttaatccccgaagttacagatatcgttgttgagtgtgcgggaataaatgcagtcaagcaacacgggatcgaagccatcaaggcaggaaaagatctctacataatcagttcgggagcgttttcagatcccaagtttcctactgagctccttaaccatcttaagagcagcacttccaaagttttcgtgccatcaggtgctatcggaggccttgatataatcagggcagtgaggacccgaatatcctctgttagactcataatgacgaagccaccttcttcactcggctataaggagcgtttctcagagccacaagtagtattcgagggacgcgttgaaaaagcaattgagagattccctcagaatgtcaatgttgcagttaccctgctgctcgcagtgggagaaagtgccaaggttacagttaaggtcgtggttgatccgacaatagatagaaatacgcatgaggtagaagtgaagtcttctgttggtgattataaaatcgttcatgaaaacaaaccgtcgccaaatctaaagacaagttatctggcagcgctctcgttggcttcgtgcataaacagaagattcgacaggttagtagtagggggttga

SEQ ID NO: 12 - DNA, 978 bp, Thermotoga maritima
atgaaagtaggagttgttggtgccacgggagaagttggaagaacgatggtaaaagtactcgaagaattcaacgttcccgtcacggagctcaggctcttcgcttcggaaagatctgtgggtaaagaaattgaattcaaaggtgagaaattcaaggtcgagcttctcacggaagaatcgatgaaatggaagtgtgactacttcctgttttccgcgggtgccagtgtttccagaaagttcgctcctatcgcagccgaaaacggagtgaccgtgatagataactcttctgctttcagaatggagaaggaaataccccttgtggttccggaggtgaacgcttaccttctcaagggatacacaggaataatagcaaatccgaactgttcaacgattcagatgatcctttccatctacaaacttcacgaagtttacggaatagaagagatctttgtgtcgacgtatcagtccgtctccggcgctggtcataaggggatagaagaactccttgctcaagaaagaggagaaaacgtgatgaaagtcttcccaaaacccattcacagaaacgtcattcctctcataggtgatatccaggaaaatcttttctctcaggaagagatgaagatggtgaatgaaacaagaaaaattctgaacgactactcgataagggtgtatccaacaacggtgagggtgcccgttctgtacggacactctgaagcgatcatggtgaggctcaagaaaccctacgagtctctcgaaaaggtgagagaagtcatagcttctggagaagacgtggtggtgacggacgatctcataacaccggtggatgtcgcaggaaagaacgaaacttatgtttgccgactcagagcgaccgatgaaagatccattcttttctggaacgtggcggacaacatccgtgtaggggctgcgaccaacgccgtcagaattctcctgaagcacgctgagatgaacggaaaggtgtga

SEQ ID NO: 13 - DNA, 783 bp, Candidatus Altiarchaeales archaeon IMC4
atgatgaagattggtataatcggctgcggtaatatcggcagggtggtcatccgggctgtttttgagggggttgttgattgtgaggttgtgtgtgtttttgatgccgatcgcagggggtttgagaagcttccgaaggaagttatatcatgtcttttgtttacggataagtttgatttttttataatgcaggatatggacattgtcgtggaggcggcatcgcaggaggcggttcgcgaattttcggcgtttgttttgggggggggtaaggatatgatgataatgagcgtcggggccttggtagatgccgggtttcgcgggcagttggttgggttggcgaaagagaagaaggttaagatatatattccctcaggtgcaatcgccggcatcgatggtcttaagtccgctatgtctgcgggggttgggggggttgtgctgacgacaagtaagcccccgtcaagccttggcgtggatacaaaaacaaaaagaattatttatgatggatatgctgaagaggcggttaggttatttccaaaaaacgttaatgtttcggccaccctcgcgctagcgggcgttggttttgaaaagacgagggttaaaataattgcagaccctaatttaaaggaaaatgttcatgaggttgttgtgcgtggcgacttcggaacttttagcgtgcgagtggaaaacgtgccgagcccggataacccaaagactagttaccttgccgcgctttccgcaatagcaaccctcaaaaaaattacttcccccttacaaatcggtacatag

SEQ ID NO: 14 - DNA, 786 bp, Mumia flava
atgaccacgtcgagtcccacccgtgaggtcgccgtgctcggcttcggctcgatcggctccgtcgtcgccgacgagctcgccgcaggacgcgtccccggcgcacgcctgagctgcgtggtcggcgatcgggcccgcggccgggtcgacgtcccggtcgtcgacgtcgacgaggcgaccgcccgtgccgacgtcctgatcgagtgcgccgggcacgccgccctgctcgcgcacggggcgcggatcctcgactccgggacggatctggtgatctcgtcggtcggcgccctcgtcgaccgcgacctccgggcccgcctggatgcggccgggccgggccgtaccttcctcacaacgggcgcgctcggcgggctcgacctgctggtggcaggcgcctccgccgctcccttcgggcgggtccggctgacgacgacgaagacgccctccgcactcgtgcaggactggatggacgacccgcagcgtgacgcgctgctcggcaccgacgcgcccgtcgtcgtcttccgcggcacggcagagcaggcggcgccgctgttccccaggtccctcaacgtcgccgcgaccctggcgctcatgctccccgagagcgaggtcgaggtggagctggtcgccgatccggccgccaccctggtgtcgcacgtggtggaggcggacgggccggtcgggacgtaccggttcgaggttcgcaaccgcccgtcgccgaccaacccgcggaccagccaggtcgtcccgtacgcggtgctgcggaccctccgccaggccctcgccgtctga

SEQ ID NO: 15 - DNA, 765 bp, Amycolatopsis thermoflava
atgatcggcgcgggctcgatcggcggcgtggtcgcccgcgccctgcgcgacggatcagtgccgggtgcgacgctctccggcgtcgtggacccggccggtgcggcggatctgccgctggtgtcgctggacgaacttctgtccacttcggacctggtagtcgaggcggccgggcagcgggcgctggcggaggtcggaccgcaggtgctggccgccgggcgggacctgctggtcgtgtcggtcggcgcgctggccgacgacgccctgctggacaagctgctgtgcgcgggccccggtgagctgcacctgtcgaccggggcgatcggcggcctggacctgctgcgggcggcggcccggatggcgccgctgacccgagtgacgatcgagaccacgaaactggccgcgaacctggttcaggcatggatgtccgacgaggaggccgcgcggctgcggaccaccgccgagccggtcgagctgatgcgcggcccggcacgcgaggtgaccgcggcgttcccgaagtcggcgaacgtggctgcctcggtggcgctggccgtgggcgactgggacgtggtggaggcggcggtgatcgccgacccggccgccgagctgacctcgcacgtcatcaccgccgacgggccggccgggtcgtaccggttcgagatccgcaaccggccctcgccgcggacgccgacgagcagtgaggtcgtgccgcacgcggtgctcgccgcgatcgccgcgctggcggagccgcgggtggtgttccggtga

SEQ ID NO: 16 - protein, 260 aa, Candidatus Hydrothermae bacterium
MRAGIIGCGAIGSFLAREIDRGNVAHMKLVALFDIDLNKVYKLVESLEHKPQIADSFEKFLKLPVDFVIEAASQQAVFQYAEKILKQKKPLLLMSAGALADDRLREKLFRVARENNTKIYIPSGAIAGLDGLKAMSNVRLHRARLTTRKSPSALGVKTEKPVVVFSGNAHEAAKRYPQNINVAIAFGLAAHAIDILQVEIVADPGVSRNIHTIEVEGEAGKLEITLENFPFPDNPKTSFLAALSALQVLKNIASNVVIGG

SEQ ID NO: 17 - protein, 263 aa, Glaciecola sp. 33A
MIKIGLIGFGAIGRCVIETLPKALTEEYEVIGILTRKAADNWVNNIPSYSDIDQLLAKQPDIIVECAGHHAVKEYGCKILEANISLVISSIGALADSVLYQQLKDSSTASKAKIYLPAGAIGGIDALVAAKLGGIHDVTYTMRKPPKAWQGSVAETVVDLNSLKQATVIFSGSAGEAATLYPKNTNVTATIALAGLGFDETKVELIADPNIIDNIHEISVSGETGYFTIVLKGKPSVYNPKTSALTAFSVTKCVADFGSSIII

SEQ ID NO: 18 - protein, 258 aa, Mesorhizobium sp. M7D.F.Ca.US.005.01.1.1
MVTLGLIGFGTISRAIVSAFPPDSCRWVALMREGARPALPANVSTVTQLDALISARPSTVVEAASQEAVAAYVPALLDAGIPTIIASIGAFSDPILAARLTDASRNSGARLVLPSGALGGLDYLRAIAALPDARVRYTSRKPPAAWKAELATLGLSAEHDAVSLFEGTPAQAAKLYPKNLNAAFAVALAAGIDKVTVSVVADPKTTGNTHEIEVESTAGTASFRLVNAPSPSNPKTSMLTALSLVAALSELLDREGCH

SEQ ID NO: 19 - protein, 266 aa, Rhodospirillaceae bacterium
MLNIGLLGLGAIGSDVLNMVREEFSNQIQIPAVLVKRPRKEKLMGHSLITNDFEEFFSKEQDIVLEVAGHSTVRHYGERILKSGVDLMVTSVGAFTDDTLYKRCIKAATTSGSRLIIPSAGIGSLDTLSAAAVGGLDSVHMIVRKDPTAWYGTHAENLFDLAALKKPTIIFEGSPREGAALYPQNVNISAAVSLAGMGLDKTRLTIIADTEIDTHVCEIHANGAFGSYTFREDLTVAETNRKTGKIVAMAVMKTIRQMVSPVLIGV

SEQ ID NO: 20 - protein, 260 aa, Bacillus kochii
MKLGLIGGGNIGKFLLQSINSDKLVDGAQFVGLYTRNQEKANELAEEYDLRSYQSIDELIASDIDVIVEAATVDVVRAHATSVLTHGKDLVVSSVGAFSDNDYFLQLETICKEQGTTIHLPSGAVGGLDILKAAKAIGALQEVSLTTTKPPHALNGVTLENKTVLFEGNAYEAIKQFPKNINVSIILSLAGLGSKETKVKIIADPKATKNSHEITAKGAFGKVKLVVENDPMPNNPKTSYLAALSVLSTLKHKDQSIKVG

SEQ ID NO: 21 - protein, 257 aa, Novosphingobium rosa
MLRIGFIGNGSIARAACAALGPDVTLCGHLARPGRSDGDLAVERLADLLDRQPDVVVECAGHEAVREHGAAVLEAGVALMVVSIGALADPALESALNDAATRSGARLILPAGAVGGIDALTAAKLGGLSSVTYRARKPAMAWAGSPAEKVVDLASLGEATTFFRGTAREAAIAFPKNSNVAATVALAGVGFDATQVELVADPHSSRNLHEICFEGADGAFRFEIEGRPSPDNPKTSLLTAHSVARELLTFAAQRKAR

SEQ ID NO: 22 - protein, 236 aa, Archaeoglobus fulgidus
MLVGLIGYGAIGKFLAEWLERNGFEIAAILDVRGEHEKMVRGIDEFLQREMDVAVEAASQQAVKDYAEKILKAGIDLIVLSTGAFADRDFLSRVREVCRKTGRRVYIASGAIGGLDAIFSASELIEEIVLTTRKNWRQFGRKGVIFEGSASEAAQKFPKNLNVAATLSIASGKDVKVRLVADEVEENIHEILVRGEFGEMEIRVRNRPMRENPKTSYLAALSVTRILRNLKEGLVV

SEQ ID NO: 23 - protein, 269 aa, Arthrobacter sp. 161MFSha2.1
MTSHRIGIIGYGAIGARVAEDISLGKVVGAELAGIISRTDNGTGRPAVERPFPSLTLEAALECCELIVECAGQSAVTEYAEKILGAGVDFLITSIGALADQDLAARLNACGPGRLFMTSGAVGGLDLLEAGAREAAYDSVVVSTTKLPETLVQPWMEQEQADGIRATTEPLEVFLGSAQEAARLFPRSLNVAAAVAEAVGDWDGVQVRLTADPKASLTSHVIEASGPSGEYRFEIRNNPSPQNPRTSGIVPFAVLRSLEAAIGERGGLV

SEQ ID NO: 24 - protein, 253 aa, Oceanotoga teriensis
MFLLNIFFIGAGNCTEIILEKMQNCIKKAYLLDYDVEKINFLKEKFHFCIESDFFISDDIDFYVECASVEAVKKYTENIIRNNKNIIILSSGAFSDFDFRNNVENILKNSRSQIFIPSGAIGGIDIINSLKDEINSITIETRKPPLSFNMINTKEELIFYGTAEEAIKNYPKNINVAITLSMAVESFDKVKVKIISDPKIIKNIHKIFIDSKAGKYEIKIENNPSNNPKTSLMAPLSVVGFLKKFNNSIKVGV

SEQ ID NO: 25 - protein, 251 aa, Marinitoga sp. 1155
MLKVFLLGAGNSAKIILDELNFEKVYVYDKNFKQFEKLKEIHNEIEYLDIKNLETTDVDYIIEVASVEALKNYGLKLLDMNKNLIVLSTGAFADKIFRYNFVKKLNNKNINVYVVSGAIGGIDLIRTISDKINTITLITRKTPKSLGIDIKKEKIIFEGNSIEAIERFPKNINVAVTLALAIKNFEKVKVKIIADPFIERNVHSIEIKSKVGNYTFKFENYPSKNPKTSYLAPLSIVGLLKNIHSKFKIGG

SEQ ID NO: 26 - protein, 248 aa, Thermotogales bacterium 46_20
MDKISVLLIGGGNIAHILLNELGHRIRKSYYHDLRKTDLEATFLESFLIPEVTDIVVECAGINAVKQHGIEAIKAGKDLYIISSGAFSDPKFPTELLNHLKSSTSKVFVPSGAIGGLDIIRAVRTRISSVRLIMTKPPSSLGYKERFSEPQVVFEGRVEKAIERFPQNVNVAVTLLLAVGESAKVTVKVVVDPTIDRNTHEVEVKSSVGDYKIVHENKPSPNLKTSYLAALSLASCINRRFDRLVVGG

SEQ ID NO: 27 - protein, 325 aa, Thermotoga maritima
MKVGVVGATGEVGRTMVKVLEEFNVPVTELRLFASERSVGKEIEFKGEKFKVELLTEESMKWKCDYFLFSAGASVSRKFAPIAAENGVTVIDNSSAFRMEKEIPLVVPEVNAYLLKGYTGIIANPNCSTIQMILSIYKLHEVYGIEEIFVSTYQSVSGAGHKGIEELLAQERGENVMKVFPKPIHRNVIPLIGDIQENLFSQEEMKMVNETRKILNDYSIRVYPTTVRVPVLYGHSEAIMVRLKKPYESLEKVREVIASGEDVVVTDDLITPVDVAGKNETYVCRLRATDERSILFWNVADNIRVGAATNAVRILLKHAEMNGKV

SEQ ID NO: 28 - protein, 260 aa, Candidatus Altiarchaeales archaeon IMC4
MMKIGIIGCGNIGRVVIRAVFEGVVDCEVVCVFDADRRGFEKLPKEVISCLLFTDKFDFFIMQDMDIVVEAASQEAVREFSAFVLGGGKDMMIMSVGALVDAGFRGQLVGLAKEKKVKIYIPSGAIAGIDGLKSAMSAGVGGVVLTTSKPPSSLGVDTKTKRIIYDGYAEEAVRLFPKNVNVSATLALAGVGFEKTRVKIIADPNLKENVHEVVVRGDFGTFSVRVENVPSPDNPKTSYLAALSAIATLKKITSPLQIGT

SEQ ID NO: 29 - protein, 261 aa, Mumia flava
MTTSSPTREVAVLGFGSIGSVVADELAAGRVPGARLSCVVGDRARGRVDVPVVDVDEATARADVLIECAGHAALLAHGARILDSGTDLVISSVGALVDRDLRARLDAAGPGRTFLTTGALGGLDLLVAGASAAPFGRVRLTTTKTPSALVQDWMDDPQRDALLGTDAPVVVFRGTAEQAAPLFPRSLNVAATLALMLPESEVEVELVADPAATLVSHVVEADGPVGTYRFEVRNRPSPTNPRTSQVVPYAVLRTLRQALAV

SEQ ID NO: 30 - protein, 254 aa, Amycolatopsis thermoflava
MIGAGSIGGVVARALRDGSVPGATLSGVVDPAGAADLPLVSLDELLSTSDLVVEAAGQRALAEVGPQVLAAGRDLLVVSVGALADDALLDKLLCAGPGELHLSTGAIGGLDLLRAAARMAPLTRVTIETTKLAANLVQAWMSDEEAARLRTTAEPVELMRGPAREVTAAFPKSANVAASVALAVGDWDVVEAAVIADPAAELTSHVITADGPAGSYRFEIRNRPSPRTPTSSEVVPHAVLAAIAALAEPRVVFR

SEQ ID NO: 31 - DNA, 35 bp, Artificial Sequence
  primer (a-1) for amplifying tac promoter
ttttataacccgggccatcgactgcacggtgcacc

SEQ ID NO: 32 - DNA, 35 bp, Artificial Sequence
  primer (b-1) for amplifying tac promoter
tgctagcactgtttcctgtgtgaaattgttatccg

SEQ ID NO: 33 - DNA, 38 bp, Artificial Sequence
  primer (a-2) for preparing multicloning site
ggaaacagtgctagcagatctggaggagaaacgcatat

SEQ ID NO: 34 - DNA, 72 bp, Artificial Sequence
  primer (b-2) for preparing multicloning site
cagtgcggccgcaagcttgtcgacggagctcgaattcggatccgatatcagcatatgcgtttctcctccaga

SEQ ID NO: 35 - DNA, 80 bp, Artificial Sequence
  primer (a-3) for preparing multicloning site
acaagcttgcggccgcactgcagcaccatcaccaccatcattgataagatccggctgctaacaaagcccgaaaggaagct

SEQ ID NO: 36 - DNA, 63 bp, Artificial Sequence
  primer (b-3) for preparing multicloning site
tatttgaatcgagttattgctcagcggtggcagcagccaactcagcttcctttcgggctttgt

SEQ ID NO: 37 - DNA, 35 bp, Artificial Sequence
  primer (a-4) for amplifying rrnB terminater
taactcgattcaaataaaacgaaaggctcagtcga

SEQ ID NO: 38 - DNA, 35 bp, Artificial Sequence
  primer (b-4) for amplifying rrnB terminater
cctagatccgcggagtttgtagaaacgcaaaaagg

SEQ ID NO: 39 - DNA, 35 bp, Artificial Sequence
  primer (a-5) for amplifying DNA replication origin of pUC19
acaaactccgcggatctaggtgaagatcctttttg

SEQ ID NO: 40 - DNA, 35 bp, Artificial Sequence
  primer (b-5) for amplifying DNA replication origin of pUC19
cgtccgcggccagcaaaaggccaggaaccgtaaaa

SEQ ID NO: 41 - DNA, 35 bp, Artificial Sequence
  primer (a-6) for amplifying nptII gene
ttgctggccgcggacgtagaaagccagtccgcaga

SEQ ID NO: 42 - DNA, 35 bp, Artificial Sequence
  primer (b-6) for amplifying nptII gene
ggcccgggttataaaagccagtcattaggcctatc

SEQ ID NO: 43 - DNA, 35 bp, Artificial Sequence
  primer (a-7) for amplifying DNA fragment of inserted pTH1
aattgtcagataggcctaatgactggcttttataa

SEQ ID NO: 44 - DNA, 35 bp, Artificial Sequence
  primer (b-7) for amplifying DNA fragment of inserted pTH1
tgacgccagaagcattggtgcaccgtgcagtcgat